European Patent Specification EP 3 980 134 B1, published July 26, 2023. Title: Bioactive peptides and compositions comprising them. Applicant: Espikem S.r.l. Università degli Studi di Firenze. The sequence listing filed with the application follows.

SEQUENCE LISTING (5 sequences)

SEQ ID NO: 1 - protein, 4 aa, Artificial Sequence
  Synthetic peptide
NVVK

SEQ ID NO: 2 - protein, 4 aa, Artificial Sequence
  Synthetic peptide
NVVK

SEQ ID NO: 3 - protein, 10 aa, Artificial Sequence
  Synthetic peptide
MGKVVNPTQK

SEQ ID NO: 4 - protein, 4 aa, Artificial Sequence
  Synthetic peptide
KVVN

SEQ ID NO: 5 - protein, 4 aa, Artificial Sequence
  Synthetic peptide
KVVN